European Patent Application EP 4 385 522 A1, published June 19, 2024. Title: Microtubule Inhibitor-Based Antibody-Drug Conjugate. Applicant: KUNSHAN XINYUNDA BIOTECH CO., LTD. The sequence listing filed with the application follows.

SEQUENCE LISTING (4 sequences)

SEQ ID NO: 1 - protein, 214 aa, synthetic construct
DIQLTQSPSSLSASVGDRVSITCKASQDVSIAVAWYQQKPGKAPKLLIYSASYRYTGVPDRFSGSGSGTDFTLTISSLQPEDFAVYYCQQHYITPLTFGAGTKVEIKRTVAAPSVFIFPPSDEQLKSGTASVVCLLNNFYPREAKVQWKVDNALQSGNSQESVTEQDSKDSTYSLSSTLTLSKADYEKHKVYACEVTHQGLSSPVTKSFNRGEC

SEQ ID NO: 2 - protein, 451 aa, synthetic construct
QVQLQQSGSELKKPGASVKVSCKASGYTFTNYGMNWVKQAPGQGLKWMGWINTYTGEPTYTDDFKGRFAFSLDTSVSTAYLQISSLKADDTAVYFCARGGFGSSYWYFDVWGQGSLVTVSSASTKGPSVFPLAPSSKSTSGGTAALGCLVKDYFPEPVTVSWNSGALTSGVHTFPAVLQSSGLYSLSSVVTVPSSSLGTQTYICNVNHKPSNTKVDKRVEPKSCDKTHTCPPCPAPELLGGPSVFLFPPKPKDTLMISRTPEVTCVVVDVSHEDPEVKFNWYVDGVEVHNAKTKPREEQYNSTYRVVSVLTVLHQDWLNGKEYKCKVSNKALPAPIEKTISKAKGQPREPQVYTLPPSREEMTKNQVSLTCLVKGFYPSDIAVEWESNGQPENNYKTTPPVLDSDGSFFLYSKLTVDKSRWQQGNVFSCSVMHEALHNHYTQKSLSLSPGK

SEQ ID NO: 3 - DNA, 642 bp, synthetic construct
  source 1..642: mol_type = other DNA
gacatccagctgacccagtccccatcttctctgtccgctagtgtgggcgacagagtgtctatcacatgcaaggcgtctcaggacgtgagcatcgccgtggcttggtatcagcagaagcccggcaaggccccaaagctgctcatctactccgcttcttacagatacaccggcgtgcccgaccggttcagcggctctggctctggcacagacttcacactgacaatctctagcttgcagcctgaggacttcgccgtgtactactgccagcagcactacatcaccccactcacattcggcgctggcaccaaggtggagatcaagagaacagtggccgctcctagcgtgttcatcttccctcctagcgacgagcagctgaagagcggcaccgcttccgtggtgtgcctgctgaacaacttctaccctcgggaggctaaggtgcagtggaaggtggacaacgcccttcaatccggcaactctcaggagtctgtgaccgagcaggactctaaggactccacatactccctgtcctccacactgacactgtctaaggccgactacgagaagcacaaggtgtacgcttgcgaggtgacccaccagggcctcagctctcctgtgacaaagtctttcaaccggggcgagtgc

SEQ ID NO: 4 - DNA, 1353 bp, synthetic construct
  source 1..1353: mol_type = other DNA
caggtgcagctccagcagtccggcagcgagctgaagaagcctggcgcttctgtgaaggtgtcttgcaaggcgagtggctacacattcaccaactacggcatgaactgggtgaagcaggctcctggccagggcctcaagtggatgggctggatcaacacatacacaggcgagccaacatacacagacgacttcaagggccggttcgctttcagcctcgacacctctgtgtctaccgcttacctacagatcagctccctgaaggccgacgacaccgctgtgtacttctgcgctagaggcggcttcggcagctcttactggtacttcgacgtgtggggccagggctctctcgtgacagtgtctagcgccagcacaaagggcccatccgtgttcccactcgctccttcttctaagtctacatctggcggcaccgccgccctcggctgcctcgtgaaggactacttcccagagcctgtgacagtgtcttggaactccggcgccctcacatccggcgtgcacacattccccgccgtgttacaatctagcggcctgtactctttaagctctgtggtgaccgtgccatctagctctctcggcacccagacctacatctgcaacgtgaaccacaagccatctaacaccaaggtggacaagagagtggagccaaagtcttgcgacaagacccacacatgcccaccttgccccgcccccgagctgctgggcggcccatctgtgttcctgttcccacctaagccaaaggacacactcatgatcagcagaacccccgaggtgacatgcgtggtggtggacgtgtctcacgaggaccccgaggtgaagttcaactggtacgtggacggcgtggaggtgcacaacgctaagaccaagccacgggaggagcagtacaacagcacctaccgggtggtgagcgtgctgaccgtgctgcaccaggactggctgaacggcaaggagtacaagtgcaaggtgtccaacaaggctctgcccgcccctatcgagaagacaatcagcaaggctaagggccagcctagagagcctcaggtgtacacactgcctccatctcgggaggagatgacaaagaaccaggtgagcctcacatgcctcgtgaagggcttctaccctagcgacatcgccgtggagtgggagtctaacggccagcctgagaacaactacaagaccacccctccagtgctcgactccgacggctctttcttcctgtactctaagctgacagtggacaagtccagatggcagcagggcaacgtgttctcttgctccgtgatgcacgaggccctccacaaccactacacccagaagtccctgtccctgtctcctggcaag